European Patent Specification EP 3 821 904 B1, published February 5, 2025. Title: FORMULA OF NEUREGULIN PREPARATION. Applicant: Zensun (Shanghai) Science & Technology, Co., Ltd. Application Divisional application based on EP 14876973.0. The sequence listing filed with the application follows.

SEQUENCE LISTING (2 sequences)

SEQ ID NO: 1 - DNA, 183 bp, Homo sapiens
agccatcttgtaaaatgtgcggagaaggagaaaactttctgtgtgaatggaggggagtgcttcatggtgaaagacctttcaaacccctcgagatacttgtgcaagtgcccaaatgagtttactggtgatcgctgccaaaactacgtaatggcgagcttctacaaggcggaggagctgtaccag

SEQ ID NO: 2 - protein, 61 aa, Homo sapiens
SHLVKCAEKEKTFCVNGGECFMVKDLSNPSRYLCKCPNEFTGDRCQNYVMASFYKAEELYQ